European Patent Specification EP 3 527 070 B1, published December 3, 2025. Title: Humanized Light Chain Mice. Applicant: Macdonald, Lynn Stevens, Sean Gurer, Cagan Hosiawa, Karolina A. Andrew J. Murphy. The sequence listing filed with the application follows.

SEQUENCE LISTING (163 sequences)

SEQ ID NO: 1 - protein, 754 aa, Mus musculus
MLSLTWGMRLVERPVVPRVLLLLFALWLLLLVPVWCSQGHPTWRYISSEVVIPRKEIYHTKGLQAQRLLSYSLRFRGQRHIIHLRRKTLIWPRHLLLTTQDDQGALQMEYPFFPVDCYYIGYLEGILQSMVTVDTCYGGLSGVIKLDNLTYEIKPLNDSQSFEHLVSQIVSESDDTGPMNAWKHWSHNTGSPSSRLEYADGAPRLSSKNYATHPAAIKGHFQATHSVYSASGGDKLSSTVEYLFKVISLMDTYLTNLHMRYYVFLMTVYTEADPFSQDFRVPGGQAHTFYERVFYAHFRPDAGAIINKNSPGDDAVNPAERSICSPSALICLGQHGRNPLFLSIIITNRVGRSLGLKHDEGYCICQRRNTCIMFKNPQLTDAFSNCSLAEISNILNTPDLMPCLFYDRHVYYNTSLTYKFCGNFKVDNNEQCDCGSQKACYSDPCCGNDCRLTPGSICDKELCCANCTYSPSGTLCRPIQNICDLPEYCSGSKFICPDDTYLQDGTPCSEEGYCYKGNCTDRNIQCMEIFGVSAKNANIKCYDINKQRFRFGHCTRAEESLTFNACADQDKLCGRLQCTNVTNLPFLQEHVSFHQSVISGVTCFGLDEHRGTETADAGLVRHGTPCSRGKFCDRGACNGSLSRLGYDCTPEKCNFRGVCNNRRNCHCHFGWSPPKCKEEGHSGSIDSGSPPVQRRIIKQNLEPVVYLRILFGRIYFLFVALLFGIATRVGVTKIFRFEDLQAALRSWQEQAKDK

SEQ ID NO: 2 - protein, 756 aa, Mus musculus
MLSLTWGMRLVERPVVPRVLLLLFALWLLLLVPVWCSQGHPTWRYISSEVVIPRKEIYHTKGLQAQRLLSYSLHFRGQRHIIHLRRKTLIWPRHLLLTTQDDQGALQMDYPFFPVDCYYIGYLEGIPQSMVTVDTCYGGLSGVMKLDDLTYEIKPLNDSQSFEHLVSQIVSESDDTGPMNAWKHWSHNTGSPSSRLEYADGAPRISSKNYATHPAAIKGHFQATNSVYNSAAGDKLSSTVGYLFQVISLMDTYLTNLHMRYYVFLMTVYTNSDPFRLEFAVPGGSAYNYYVSVFYNKFKPDAGVLLNKYGPQDNQVNPAERSICSSLALICIGKYDRNPLFLSPIITNRVGRSLGLKYDEGYCVCQRRNTCIMFRHPQLTDAFSNCSLAEISNILNTPGLMPCLFYDRHVYYNTSLTYKFCGNFKVDNDEQCDCGSQKACYSDPCCGNDCRLTPGSICDKELCCANCTYSPSGTLCRPIQNICDLPEYCNGTKYICPDDTYLQDGTPCSEDGYCYKGNCTDRNIQCMEIFGVSAKNANIKCYDINKQRFRFGHCTRAEESLTFNACADQDKLCGRLQCTNVTNLPYLQEHVSFHQSIISGFTCFGLDEHRGTETTDAGMVRHGTPCSKSKFCDQGACSGSLSHLGYDCTPEKCSFRGVCNNHRNCHCHFGWKPPECKEEGLSGSIDSGSPPVQRHTIKQKQEPVVYLRILFGRIYFLFVALLFGIATRVGVTKIFRFEDLQATLRSGQGPARDKPK

SEQ ID NO: 3 - DNA, 13894 bp, Artificial Sequence
  synthetic
gtcctaaggtagcgagggatgacagattctctgttcagtgcactcagggtctgcctccacgagaatcaccatgccctttctcaagactgtgttctgtgcagtgccctgtcagtggaaatctggagagcatgcttccatgagcttgtgagtagtatatctagtaagccatggctttgtgttaatggtgatgttctacataccagttctctggcttaataatgaggtgatgattctatgttcctgtaacgcttcctcaactgggtcctaagtctttcttcactccatctattcctctaaggaatgatcctgaaaatcccatcacaaactataggagatgggaaccatcaaaaaacacagtgacaaagaggtgggaacgcatcagggttcaggaaccatattttaaaaagatatcgtaaataacttcttaaaagagatatagacaaatctccattaatacggagaccagaggcctaaggctaagaaccaatggtggctcaaggtctcctgctacccgaggagcaaacgtagagcagtttctaatgatttatttaaaatatagaatcaaaagtaccagtttgcaattttgaaagatttatttcagcaatgcaacaacatcaggtggtgccgagtccaacacgtcttatgtcccatgatataaacaaaggccatccagaactgtggactggagttctaccttgtcccctaatgacattcagattttttttccattctctttatcttagaggagacagggggctaactcattttacttgtcctttgcttgttcttgccaagaacgtaaagcagcttgcaagtcttcaaacctaaatatcttagtaactcctacacgagtggcaatgccaaagagcagtgcaacaaagaggaagtaaatacgaccaaagagtattcttaaatacactactggctctaggttctgttttattatgcgcctttgaaccggaggggacccactgtctatgctcccactgtgtccctcttctttgcactttggagggctccaaccaaaatggcaatggcaattccgacgattgttacacactcctctgaaattgcatttttctggggtgcagtcataacccaaacgagataaacttccattgcaagctcctcgatcacagaacttaccccttgaacacggggtaccatgtctcaccaatccagcatctgctgtttctgtcccacgatgttcatcaagcccaaagcaggtaaccccagagataaccgattgatggaatgaaacatgttcttgcaaaaatggaagattggtgacattggtacactgcaaccttccacacagcttgtcctgatcagcacaagcattgaatgtgaggctttcttctgctctagtacaatgcccaaatcgaaaccgttgtttgttgatgtcatagcacttaatattagcattcttagcacttacaccaaagatttccatgcattgtatgttgcgatcagtgcagttacctttatagcagtaaccctcttctgagcatggtgtcccatcttgcagataagtgtcatctgggcaaatgaacttagagccactacagtactctggaagatcacatatgttctggataggtctgcagagtgtcccagaaggactgtaagtgcaatttgcacagcataattctttatcacaaatgctaccaggtgttaacctgcaatcatttccacagcagggatctgaataacatgccttttgggagccacagtcacactgctcattgttatctactttgaagtttccacaaaacttataagtcaatgatgtattataataaacatgacggtcatagaaaagacatggcatcagatcaggagtattaagtatgttgcttatctctgcaagggaacaattgctgaaagcatctgttaattgaggatttttgaacatgatgcaggtgttccttctctggcagatacagtacccctcatcatgttttaggcctaaactccttccaacacgattggttattataatagataaaaataaaggatttcgaccatgttgaccaagacaaattagggctgagggagaacatatactcctctcagctggattaacagcatcatctcctggcgaattcttgttaattatagctcctgcatcaggcctaaaatgagcataaaatactctctcatagaaagtatgagcctgccctcctggaactcgaaaatcttgtgaaaatggatcagcctcggtatacacagtcatgagaaagacatagtaccgcatatgaagattggtcagataggtgtccattaaactaatgactttaaacaaatactcaacagtagatgaaagtttgtcacctccagaagcactatatacagaatgggttgcttgaaagtggccttttatagcagctggatgtgtagcgtaattcttactagatagtctgggagctccatctgcatattccaatctggaggagggagaacctgtattatggctccagtgcttccatgcattcataggccctgtgtcatcagactcagatactatctgagaaacaaggtgttcaaagctctgtgaatcattgaggggtttgatttcataggtaaggttatccaactttatgacccctgacaggcccccataacaagtatccacagtgaccatggattgcaggatcccctccaggtagccaatatagtaacaatctacaggaaaaaaggggtactccatctgtaaggctccttggtcatcttgagttgtcagcaacaagtgtctgggccaaatgagtgtctttctccgcaggtggatgatatgtctctggccccgaaaacgcaagctatacgagagcagtctttgtgcttgaagtcctttggtatggtagatctccttccgaggaataaccacctccgatgagatgtaacgccaagtgggatggccttgagaacaccagactggaaccaggaggagcagccagagtgcaaatagcaagaggaggaccctggggaccacaggtctttccactagcctcatgccccaggtcagagataacatcctgggtggagctaactccctctgctgtggccactgcctggtctagaaaatactgacagaggactaaaaacctcctcaggctcccaacctaagtggttacccagacaactggagttaggtaacagtcactgggtgtggcaggaattgagtctgaatgtgttagctgaggttgaggttaaatattgtcaaaagggatgtctataaatgtgcctggacaagaaaagtcagaagcagcaaggagtgtctctgacaggctcaatcctttcttttctttttttgaagttcaaaatatcatttccacgtgaatgtatttggttcccagtgtgactctgggtctctttctaggagtcaatatttctttatatcttggctcatgtttttcacagttgttctaacttcttgttttgttttgtttgtttgtttgtttgaaagttagaagtaaatactgtctatattagccttttagctataaatgattgtttttatttcttctaatcatgttttgtttgagttttggttaaactatttacaaatgagttttttttttccttttgggtgttgctcgaaagtttggagctttctgttaatattgtgttgttgtttctccaatattattagacctgagaattctacctgggtacctgtgaactccagaatttttaaaaattccatctcttgggaacattatctctgaccccgtctgaggccgaagtggctgtccccctccaacctttagtatctttctttcctgactattgggatttcttcaagcaatcaggctgatgggttctcagcagtgagaccagtagactgtcggtatgaacgtcgaagagtctgccacacactccgggttcatcaacagtgctttcgcgtctcttacttttgtagaaggaaatgcagcctctgagttttctccaagaaatcattgatgaaagggtgaaaagatgggtatcacccggagttcatgacaagccctggctcagacacgtgagcaaggtctacagccccaaagataggctgccctgcaacatgtatttataagataggagaaaaaaatgggtagttggagggttgatcaacttacttcctctcaaacatatatatctcatctaagtgtgcaggggaaaactctgtagaactactgggatacctgctcacccccaggagcctcatgaataagtctctgcttctgccttgtagccatgagcattactgcacctgatacccctgcagcttcctagggaagagggaggaagtgacttggcccctgtctggttaaggtaagaggagataaatcccttctcattgattagggtgagaggggtcatgtgctctatcattggtgacccagttgggacatgggtttataccaaagtcatcactctgaggttctgtgtaccaccaggctgaactcccatatcctacatggacataggacaacaccaagcagaaggaggttttaggactaaactgaaggacagagatgcggtttctaaacaactagggagtgccagggccagcctctctaaccactataggacactgtggagtctggttacaaagagagattactcaaggtccttagcactgattacagagcatatctcagatgccttctgctgaccagatgtatctttgcataatctgcctatccagattcagaaaattgatgccacatagccaagtggactttcaggaacagacgatttaaaaacaggcagagagatgtgagagaaaggagaaggagagagagaagggagagggagagaagagagagggagacggagaaggaaagagggagaaggagaaggagagaaggggcatggacagagggagggacagaaggagagaggagatagagagggggataaggaagaagggagggagggagagagagagaaggctaagtctttccatacctgggtcccaatacctcttataacccaagcacatggtttcacatatcacaatgcggttgggatatagataactgtaaatacttgtgaaaataatggggctgagatctggggttttcatgatagtttcaaagtcaccgtactgactaaaaccttccactggcccatctccagcttcctaatctgagggtatcaaatttcccactaagtgtgtttagaaagatctccacctttttgcccttgtcttccagtgccccacctacgttctggtctcccacatctgatgtcttctcagtgattctggccctgcctgctccacagctacaaaccccttcctataatgagctctgtgctgagccatcatcctgaatcaatccaccttaagcagatgttttgcttatttttcctgtgtccatactacagaggaaaggtaggcatgtagaagctgaagcatctcacctcattccaagcaccctcagtctctaaatgtgcccccttgtttccagaagtgcaacctcaagcatcttttattcattcatcttagagggccacatgtgctgtagtgttataagatgaaatttaaagcattaattattcctaacaagccaattaaacaagccaaaaacattcatcagtcattcccatggaacctctgaagcatcttcctgctctaaccttgggttttccagggctgctctgggatcacaggagctgtcctgtctaccagccatataaaggcagacctatcagaattacaccagacttctcaccatagactataaaagccagaatatcctggacagatgttatacagaaactaagagaacacaaatgccagcccaggctactatacccagcaaaactctcaattaccatcgatgaagaaaccaagatattccattacaagtccaaatttacacaatatctttccataaatccagccctacaaaggatagcagatggaaaactccaacacaggtaggaaaactacaccctagaaagagcactaaagtaatcatctttcaacacactcaaaagaagataaccacacaaacataattccacctctaacaacaaaaataaagtaggcaacaatcactattccttaatatctcttttaacatcaatggactcaattctccaataaaaagacatagactaacagactgaatacataaacaggacacagcattttgctgcataaagcaaacacagcgttacttttttttttctaaatgacattttttattagatattgtctttattgacatttcaaatgttatcccctttcctggtttaccctctgaaatcccctatctcctccccctccccctgctcaccaatccacccactcccacttccaggccctggcaatcccctatatttgggcatagagccttcacaggaccaaggtactctccttgcattgatgaccaactagtccattctctgctacaaatgcagctagatctatgagtcccaccatgttttcttttgttggtggtttcatgccagggagctcttggagtactgattggttcatattgttgttctccctatggggttacaaaacccttcaacttcttgggtcctttctctggctgcctcattggggaccttgtgcgaagtccaatggatgactgtgagcatccacttctgtatttgccaggcactggcagagcctctcagaagacagctatatcaagatcctggcagcaagctcttgttggtatccacaaaagtgtctggtggttgtctatgggatggatccccaaaggggcagtctctggatggtcattccttcagtctctgttccacactttgtctctttaactccttccatgactattttattcctccctctaagaaggaccgaagtattcatactttggtcttccttcttgaaattcatgtgttttgtgaattgtatctttgatattccgaacttctgggctaatatccacttatcagtgagtgaatatcatgtgtgttcttatgtgattgagttacctcactcaggatgatatcctccagaaccatccatttgtctaagaatttaatgaattcattgtttttaatagctgaggagtactccattgtgtaaatgtaccacattttctgtacccattgttctcttgagggacatctgggttctttaaagcttctggacattaaatataaggctgctatggaaatagtggagaatgtgtccttattacatgttggagcatcttctgggtatatgcccaggagtgctattgctggatcctctgatagtactatgtccaattttctgaggaactgccaaactgatttacagagtggttgtaccagcttgcaattccaccagcaatggagaaatgttccccttcctccacatcctcaccaacatctgctgtcacctcaatttgttcttagtgattcagacaggtgtgaggtggaatatcagggttgtttggcatttccctgatgactagtgatattgaaaaaaattttaagtgtttctcagccattcagtattcttcagttgagaattcactgtttagctctgtactcaggtttttttaatagggttatttggttttctggagtctaacgtcttgaattctttctatatattggatattagccctctgtcatatttaggattggtaaagatctttcccaatatgttggctgcctttttgtgtcctttgccttacagaacctttttaattttatgaggtcccatttgctaattcttcattttacagcacaagccattggtgttctgttcaaaaatctttccccctgaaccctatcttcgaggatcttccccactttctcctctataagtttcagtgtctctattattgtgctgaggggtaccgaagttcctattccgaagttcctattctctagaaagtataggaacttccctagggtttaaacccgcggtggagctctgatgtgggaacgcttcagtgttcaggaaccatatgatttatttaaaatatagaatcaaaagtaccaatttgcagttttgaaagatttattccagtgtaagcattagcaatgcaccaacatcaggtgatttctgaatccaacacgtcttatgtcctcatgatattaaaaaaaaaaaaaggccatccagaactgtgaacttgagttctaccttgttccctactgacattcagattttcttttttgcattctctttatcttacaggagacaggaggggagggctaactcattttactttggcttgtcccttgctggtccttgcccagaacgtaaagtagcttgcaagtcttcaaatctaaaaatcttagtaactcctacacgagtggcaatgccaaagagcagtgcaacaaagaggaagtaaatacgaccaaagagtattcttaaatacaccactggctcttgtttttgttttattgtgtgcctttgaactggaggggacccactgtctatgctcccacttagtccctcttctttgcactctggaggcttccaaccaaaatgacaatggcaattccgatgattgttacacactcctctaaaactgcatttttctggggtgcagtcataacccaaatgagataaacttccactgcaagctccttgatcacagaacttacttttggagcagggggtaccatgtctcaccattccagcatctgttgtttctgtcccacgatgttcatcaagcccaaagcaggtaaacccagagataatcgattgatggaatgaaacatgttcttgcaaatatggaagattggtgacattggtacactgcaaccttccacacagcttgtcctgatcagcacaagcattgaatgtgaggctttcttctgctctagtacaatgcccaaatcgaaaccgttgtttgttgatgtcatagcacttaatattagcattcttagcacttacaccaaagatttccatgcattgtatgttgcgatcagtgcagttacctttatagcagtaaccatcttctgagcatggtgtcccatcttgcagataagtgtcatctgggcaaatgtatttagtcccattacagtactctggaagatcacatatgttctggataggtctgcagagtgtcccagaaggactgtaagtgcaatttgcacagcataattctttatcacaaatgctaccaggtgttaacctgcaatcatttccacagcagggatctgaataacatgccttttgggagccacagtcacactgctcatcgttatctactttgaagtttccacaaaacttataagtcaatgatgtattataataaacatgacggtcatagaaaagacatggcatcagaccaggagtattaagtatgttgcttatctctgcaagggaacaattgctgaaagcatctgttaattgaggatgtctgaacataatgcaggtgttccttctctggcagacacagtacccctcatcatattttaagcctaaactccttccaacacgattggttattataggagataaaaataaaggatttcgatcatatttaccaatacaaattagggctaaggaagaacatatactcctctcagctggattaacctggttatcttgtggcccatacttattaagtaaaactcctgcatcaggcttaaatttattataaaagactgacacatagtaattataagccgaccctcctggaactgcaaactcaagtcgaaatggatcagaattggtgtacacagtcatgagaaagacatagtaccgcatatgaagattggtcagataggtgtccattaaactaatgacttgaaacaaatacccaacagtagatgaaagtttgtcacctgcagcagaattatatacagaattggttgcttgaaagtggccttttatagcagctggatgtgtagcgtagttcttactagatattctgggagctccatctgcatattccaatctggaggagggagaacctgtattatggctccagtgcttccatgcattcataggccctgtgtcatcagactcagatactatctgagaaacaaggtgttcaaagctctgtgaatcattgaggggtttgatttcataggtaaggtcatctaacttcatgacccctgacaggcccccataacaagtatccacagtgaccatggattgtgggatcccctccaggtagccaatatagtaacaatctacaggaaaaaaggggtaatccatctgtaaggctccttggtcatcttgagttgtcagcaacaagtgtctgggccaaatgagtgtctttctccgcaggtggatgatatgtctctggccccgaaaatgcaagctatatgagagcagtctttgtgcttgaagtcctttggtatggtagatctccttccgaggaataaccacctccgatgagatgtaacgccaagtaggatggccttgagaacaccagactggaaccaggaggagcagccagagtgcaaatagcaagaggaggaccctggggaccacaggtctttccactagcctcatgccccaggtcagagataacatcctgggtggagctaaatccctctgctgtggccactgcctggtctagaaaatactgacagaggactaaaaacctcctcaggctcccaacctaagtggttacccagacaactggagttaggtaacagtcactgggtgtggcaggaattgagtctgaatgtgttagctgaggttgaggttaaatattgtcaaaagggatgtctataaatgtgcctggacaagaaaagtcagaagcagcaaggagtgtctctgacaggctcaatcctttcttttctttttttgaagttcaaaatatcatttccacgtgaatgtatttggttcccagtgtgactctgggtctctttctaggagtcaatatttctttatatcttggctcatgtttctcacagttgttctaatttcttgttttgttttgtttgtttgtttgaacgttagtagtaaatactgtctatattagccttttagctataaatgattgtttttatttcttctaatcatattttgtttgagttttggttaaactatttacaaatgagttttttttttttccttttgggtgttgctcgaaagtttggagctttctgttaatattgtgttgttatttttccaatattattagacctgagaattctatctgggtacctgtgaactctagaatttttaaaaattccatctcttgggaacattacctctgaccccgtctgaggccgaagtggctgtccccctccaacctttagtatctttctttcctgactattgggatttcttcaagcaatcaggctgatgggttctcagcagtgagaccagtagactgccggtatgaacgtcgaagagactgccacacactccaggttcatcaacagtgctttcgcgtctcttacttttgtagaaggaaaagcagcctctgagttatctccaagaaatcattaatgaaagagttaaaagatgggtatcacccggagttcatgacaagccctggctcagacacgtgagcaaggtctacagccccaaagataggctgccctgcaacatgtatttataagatagaagaaaaaaatgggtggttggagggttgatcaacttacttcctctcaaacatatatatctcatctaagtgtgcaggggaaaactctgtaggactactgggattgttattatcattattattattattattattattattattattattattattattaacttaaggcattttattagatattttcttcatttagttttcaaatgttatccccggaacctcctatactctctccctgccctgctccccaacccacccactcctacatcctggccctggcattcccctatactgtggcagatgatcttcgtaagaccaagagcctttcctcccattgatggcctactaggctatcctcttttacatatgcaactagagtcacagctctggggaggtattgcttagttcatattgtttttcctcctatagggttgcagatccctttagctccttgggtactttctctagctcctccattgggggccctgtgttccatccaatagatgactgtgagcatccacttctgtatttgccaggtattggcatggatcttactgcaccttctgaactctctaagcagctttcctggtcacctccaggagcctcatgaataagtctctgcttcccccttgtggctatgagcattactgcacctgatacaccctgcagcttcctagggaagagggaggaagtggcttggcccctgtctggttaaggtaagaggagataaatcccttctcatgaattagggtgagaagggtcatgtgctctatcattggtgaccaacttggggacatgggcttatacagtcatcactctgaggctctgtgtaccaccagactgaactcccatatcctacatgcacataggacaacaccaagtagaaggaggttttaggactaaactgaaggacagagatggggtttctaaacaactagggagtgccagggccagcctctctaaccactataggacactatggagtctggttacaaagagagattactcaaggtccttagcactgattacagagcatatctcagatgccttctgctgaccagatgtatctttgcataatctgcctatccagattcagaaaattgatgccacatagccaagtggactttcaggaacagacgatttaaaaacaggcagagagatgtgagagaaaggagaaggagagagagaagggagagggagagaagagagagggagacggagaaggaaagagggagaaggagaaggagagaaggggcatggacagagggagggacagaaggagagaggagatagagagggggataaggaagaaaggagggagggagagagagagaaggctaagtctttccatacctgggtcccaatacctcttataacccaagcacatggtttcagatatcacaatgcggttgggatatagataactgtaaatacttgtgaaaataatggggctgagatctggggttttcatgatagtttcaaagtcactgtactgactaaaaccttccactggcccatctccagcttgttaatctgagggtatcaaatttcccactaagtgtgtttagaaagatctccacctttttgccctagtcttccagtgccccacctacgttctggtctcccacatctgatgtcttctcagtgattctggccctgcctgctccacagctacaaaccccttcctataatgagctctgtgctgagccatcatcctgaatcaatccaccttaagcagatgttttgcttatttttcctgtgtccatactacagaggaagggtaggcatgtagaagctgaggcatctcatctcactctaagcaccctcagtctctaaatgtgcccctttgtttccagcagttcagcctcaagcatcttttattcactcgtcttagagggacacatgtgctgtagtgttataagatgaaatttaaagcattagttattcccaacaagccaattaaacaagccaaaaacattcatcagtcattcccatggaacctctgaagcatcttcctgctctaaccttgagtttcctagggctgctgtgggatcacaggagctgtcctgtttaccagcctatcctgtcccacgggattcagttattagtgggtgcgagggggaccgcaaacctggaagaaaatgggattggaagagaaaagagaaacgaagaccaagtagatcttttcctatcaaggtcttcgtttattaggctgaggtgcctggtgtaaagcatgcatcgcggggaataggaaggggtcgagggggaattttacaaagaacaaagaagcgggcatctgctgacatgagggccgaagtcaggctccaggcagcgggagctccaccgcggtggcgccatttcattacctctttctccgcacccgacatagataaagctta

SEQ ID NO: 4 - DNA, 251 bp, Artificial Sequence
  synthetic
ccagcttcattagtaatcgttcatctgtggtaaaaaggcaggatttgaagcgatggaagatgggagtacggggcgttggaagacaaagtgccacacagcgcagccttcgtctagacccccgggctaactataacggtcctaaggtagcgaggggatgacagattctctgttcagtgcactcagggtctgcctccacgagaatcaccatgccctttctcaagactgtgttctgtgcagtgccctgtcagtgg

SEQ ID NO: 5 - DNA, 245 bp, Artificial Sequence
  synthetic
aggggtcgagggggaattttacaaagaacaaagaagcgggcatctgctgacatgagggccgaagtcaggctccaggcagcgggagctccaccgcggtggcgccatttcattacctctttctccgcacccgacatagataaagcttatcccccaccaagcaaatccccctacctggggccgagcttcccgtatgtgggaaaatgaatccctgaggtcgattgctgcatgcaatgaaattcaactag

SEQ ID NO: 6 - DNA, 21 bp, Artificial Sequence
  synthetic
caggtacagctgcagcagtca

SEQ ID NO: 7 - DNA, 21 bp, Artificial Sequence
  synthetic
ggagatggcacaggtgagtga

SEQ ID NO: 8 - DNA, 17 bp, Artificial Sequence
  synthetic
tccaggactggtgaagc

SEQ ID NO: 9 - DNA, 24 bp, Artificial Sequence
  synthetic
tagtcccagtgatgagaaagagat

SEQ ID NO: 10 - DNA, 24 bp, Artificial Sequence
  synthetic
gagaacacagaagtggatgagatc

SEQ ID NO: 11 - DNA, 17 bp, Artificial Sequence
  synthetic
tgagtccagtccaggga

SEQ ID NO: 12 - DNA, 28 bp, Artificial Sequence
  synthetic
aaaaattgagtgtgaatggataagagtg

SEQ ID NO: 13 - DNA, 21 bp, Artificial Sequence
  synthetic
aaccctggtcagaaactgcca

SEQ ID NO: 14 - DNA, 19 bp, Artificial Sequence
  synthetic
agagaaacagtggatacgt

SEQ ID NO: 15 - DNA, 22 bp, Artificial Sequence
  synthetic
aactacgcacagaagttccagg

SEQ ID NO: 16 - DNA, 18 bp, Artificial Sequence
  synthetic
gctcgtggatttgtccgc

SEQ ID NO: 17 - DNA, 16 bp, Artificial Sequence
  synthetic
cagagtcacgattacc

SEQ ID NO: 18 - DNA, 19 bp, Artificial Sequence
  synthetic
tgagcagcaccctcacgtt

SEQ ID NO: 19 - DNA, 23 bp, Artificial Sequence
  synthetic
gtggcctcacaggtatagctgtt

SEQ ID NO: 20 - DNA, 18 bp, Artificial Sequence
  synthetic
accaaggacgagtatgaa

SEQ ID NO: 21 - DNA, 33 bp, Artificial Sequence
  synthetic
gctagtagtggggcctacaggccttttgatatc

SEQ ID NO: 22 - DNA, 48 bp, Artificial Sequence
  synthetic
gcaaaagcccaggggagtgggagctactacacctatgcttttgatatc

SEQ ID NO: 23 - DNA, 42 bp, Artificial Sequence
  synthetic
gcgagagagggtatagtgggaactactgaggactttgattac

SEQ ID NO: 24 - DNA, 33 bp, Artificial Sequence
  synthetic
gcgagagggacagtgggagccctctttgactac

SEQ ID NO: 25 - DNA, 36 bp, Artificial Sequence
  synthetic
gcgaaacctagtgggagctactcctggttcgacccc

SEQ ID NO: 26 - DNA, 45 bp, Artificial Sequence
  synthetic
gcgagaggaggagggtataactggaactcgaatgcttttgatatc

SEQ ID NO: 27 - DNA, 33 bp, Artificial Sequence
  synthetic
gcgagaggatataactggaactactttgactac

SEQ ID NO: 28 - DNA, 39 bp, Artificial Sequence
  synthetic
gcgaaagagtataactggaaccactggtactttgactac

SEQ ID NO: 29 - DNA, 33 bp, Artificial Sequence
  synthetic
gcgagagagataactggaaccccctttgactac

SEQ ID NO: 30 - DNA, 39 bp, Artificial Sequence
  synthetic
gcgaggggatataactggaacttttctttttttgactac

SEQ ID NO: 31 - DNA, 36 bp, Artificial Sequence
  synthetic
gcgagaggtaactggaactctctgggctttgactac

SEQ ID NO: 32 - DNA, 39 bp, Artificial Sequence
  synthetic
gcgaaaagggctactatggttcggggagctcttgactac

SEQ ID NO: 33 - DNA, 60 bp, Artificial Sequence
  synthetic
gcgagagatattactatggttcggggagttattataacgaaggtctacggtatggacgtc

SEQ ID NO: 34 - DNA, 27 bp, Artificial Sequence
  synthetic
gcgagagagtatagcagctttgactac

SEQ ID NO: 35 - DNA, 33 bp, Artificial Sequence
  synthetic
gcgagagagagtatagcagctcgttgtgactac

SEQ ID NO: 36 - DNA, 42 bp, Artificial Sequence
  synthetic
gcaagagaggataggagctcgcccctcgggtactttgactac

SEQ ID NO: 37 - DNA, 24 bp, Artificial Sequence
  synthetic
gcgagagatcttggggaaggctac

SEQ ID NO: 38 - DNA, 30 bp, Artificial Sequence
  synthetic
accacccataactggggagggtttgactac

SEQ ID NO: 39 - DNA, 18 bp, Artificial Sequence
  synthetic
gcgagagataggggaccg

SEQ ID NO: 40 - DNA, 30 bp, Artificial Sequence
  synthetic
caacagagttatagtacccctccggagacg

SEQ ID NO: 41 - DNA, 27 bp, Artificial Sequence
  synthetic
caacagcttaatagttaccctcggacg

SEQ ID NO: 42 - DNA, 26 bp, Artificial Sequence
  synthetic
caacagcttaatagttaccattcact

SEQ ID NO: 43 - DNA, 27 bp, Artificial Sequence
  synthetic
caacattttaatagttacccgctcact

SEQ ID NO: 44 - DNA, 27 bp, Artificial Sequence
  synthetic
cagcagtataataactggcctctcact

SEQ ID NO: 45 - DNA, 27 bp, Artificial Sequence
  synthetic
ctacagcataatagttacccgtggacg

SEQ ID NO: 46 - DNA, 27 bp, Artificial Sequence
  synthetic
ctacagcataatagttaccctcggacg

SEQ ID NO: 47 - DNA, 27 bp, Artificial Sequence
  synthetic
cagcagtatggtagctcacctcggacg

SEQ ID NO: 48 - DNA, 27 bp, Artificial Sequence
  synthetic
atgcaaggtacacactggccgtggacg

SEQ ID NO: 49 - DNA, 27 bp, Artificial Sequence
  synthetic
atgcaaggttcacactggccgtacact

SEQ ID NO: 50 - DNA, 27 bp, Artificial Sequence
  synthetic
atgcaaggtacacactggccgctcact

SEQ ID NO: 51 - DNA, 27 bp, Artificial Sequence
  synthetic
caacagtatgataatctccctcccact

SEQ ID NO: 52 - DNA, 27 bp, Artificial Sequence
  synthetic
caacagtatgataatctcccattcact

SEQ ID NO: 53 - DNA, 27 bp, Artificial Sequence
  synthetic
caacagtatgataatctccccgtcact

SEQ ID NO: 54 - DNA, 27 bp, Artificial Sequence
  synthetic
caacagtatgataatctcccgatcacc

SEQ ID NO: 55 - DNA, 24 bp, Artificial Sequence
  synthetic
caacggatttacaatgccgacacc

SEQ ID NO: 56 - DNA, 30 bp, Artificial Sequence
  synthetic
caacagagttacagtacccccatgtacact

SEQ ID NO: 57 - DNA, 27 bp, Artificial Sequence
  synthetic
caacagagttacagtacccctctcact

SEQ ID NO: 58 - DNA, 27 bp, Artificial Sequence
  synthetic
caacagagttacagtactcctcccact

SEQ ID NO: 59 - DNA, 219 bp, artificial sequence
  synthetic
actttcagaatgttcttgaacagtctctgagaaacacggaagacggccgcataacttcgtatagtatacattatacgaagttattctagacccccgggctcgataactataacggtcctaaggtagcgactcgagataacttcgtataatgtatgctatacgaagttatccatggtaagcttacgtggcatacagtgtcagattttctgtttatcaagc

SEQ ID NO: 60 - DNA, 21 bp, artificial sequence
  synthetic
agctgaatggaaacaaggcaa

SEQ ID NO: 61 - DNA, 19 bp, artificial sequence
  synthetic
ggagacaatgccccagtga

SEQ ID NO: 62 - DNA, 21 bp, artificial sequence
  synthetic
tcccatagggctaggatttcc

SEQ ID NO: 63 - DNA, 19 bp, artificial sequence
  synthetic
tcccctcacactgttcccc

SEQ ID NO: 64 - DNA, 19 bp, artificial sequence
  synthetic
ggtggagaggctattcggc

SEQ ID NO: 65 - DNA, 17 bp, artificial sequence
  synthetic
gaacacggcggcatcag

SEQ ID NO: 66 - DNA, 21 bp, artificial sequence
  synthetic
tcaacctttcccagcctgtct

SEQ ID NO: 67 - DNA, 24 bp, artificial sequence
  synthetic
ccccagagagagaaaacagatttt

SEQ ID NO: 68 - DNA, 20 bp, artificial sequence
  synthetic
ccctggtgaagcatgtttgc

SEQ ID NO: 69 - DNA, 20 bp, artificial sequence
  synthetic
tgtggcctgtctgccttacg

SEQ ID NO: 70 - DNA, 21 bp, artificial sequence
  synthetic
cacacctagaccccggaagtc

SEQ ID NO: 71 - DNA, 21 bp, artificial sequence
  synthetic
tcgctttgccagttgattctc

SEQ ID NO: 72 - DNA, 17 bp, artificial sequence
  synthetic
tgcggccgatcttagcc

SEQ ID NO: 73 - DNA, 18 bp, artificial sequence
  synthetic
ttgaccgattccttgcgg

SEQ ID NO: 74 - DNA, 20 bp, artificial sequence
  synthetic
gcaaacaaaaaccactggcc

SEQ ID NO: 75 - DNA, 19 bp, artificial sequence
  synthetic
ggccacattccatgggttc

SEQ ID NO: 76 - DNA, 22 bp, artificial sequence
  synthetic
ccatgactgggcctctgtagac

SEQ ID NO: 77 - DNA, 25 bp, artificial sequence
  synthetic
caagtcagggtgctaatgctgtatc

SEQ ID NO: 78 - DNA, 19 bp, artificial sequence
  synthetic
cacagcttgtgcagcctcc

SEQ ID NO: 79 - DNA, 22 bp, artificial sequence
  synthetic
gggcactggatacgatgtatgg

SEQ ID NO: 80 - DNA, 21 bp, artificial sequence
  synthetic
tcataggtaggtctcagtttg

SEQ ID NO: 81 - DNA, 21 bp, artificial sequence
  synthetic
tgatctgcgctgtttcatcct

SEQ ID NO: 82 - DNA, 31 bp, artificial sequence
  synthetic
tgacatgaaccatctgtttctctctcgacaa

SEQ ID NO: 83 - DNA, 29 bp, artificial sequence
  synthetic
agagacgctccgaggtcaaggtgctctag

SEQ ID NO: 84 - DNA, 23 bp, artificial sequence
  synthetic
tgggcacaacagacaatcggctg

SEQ ID NO: 85 - DNA, 16 bp, artificial sequence
  synthetic
accctctgctgtccct

SEQ ID NO: 86 - DNA, 26 bp, artificial sequence
  synthetic
ccaagcaggaggtgctcagttcccaa

SEQ ID NO: 87 - DNA, 24 bp, artificial sequence
  synthetic
tccacactgtcggctgggagctca

SEQ ID NO: 88 - DNA, 21 bp, artificial sequence
  synthetic
acgagcgggttcggcccattc

SEQ ID NO: 89 - DNA, 37 bp, artificial sequence
  synthetic
ctgttcctctaaaactggactccacagtaaatggaaa

SEQ ID NO: 90 - DNA, 27 bp, artificial sequence
  synthetic
tgccgcttatacaacactgccatctgc

SEQ ID NO: 91 - DNA, 37 bp, artificial sequence
  synthetic
agaagaagcctgtactacagcatccgttttacagtca

SEQ ID NO: 92 - DNA, 21 bp, artificial sequence
  synthetic
gggctacttgaggaccttgct

SEQ ID NO: 93 - DNA, 23 bp, artificial sequence
  synthetic
gacagcccttacagagtttggaa

SEQ ID NO: 94 - DNA, 23 bp, artificial sequence
  synthetic
aagaccaggagctctgcctaagt

SEQ ID NO: 95 - DNA, 22 bp, artificial sequence
  synthetic
cccatcacgaactgaagttgag

SEQ ID NO: 96 - DNA, 20 bp, artificial sequence
  synthetic
cagggcctccatcccaggca

SEQ ID NO: 97 - DNA, 28 bp, artificial sequence
  synthetic
ccccagtgtgtgaatcactctaccctcc

SEQ ID NO: 98 - DNA, 20 bp, artificial sequence
  synthetic
cctctcctcctcaccctcct

SEQ ID NO: 99 - DNA, 20 bp, artificial sequence
  synthetic
  variation (4)...(4): r=a or g
  variation (9)...(9): s=c or g
  variation 11, 12, 13: y=c or t
atgrccdgstyyyctctcct

SEQ ID NO: 100 - DNA, 18 bp, artificial sequence
  synthetic
ctcctcactcagggcaca

SEQ ID NO: 101 - DNA, 20 bp, artificial sequence
  synthetic
  variation (18)...(18): s=c or g
atggcctgggctctgctsct

SEQ ID NO: 102 - DNA, 19 bp, artificial sequence
  synthetic
  variation (11)...(11): y=c or t
  variation (13)...(13): s=c or g
atggcctggaycsctctcc

SEQ ID NO: 103 - DNA, 23 bp, artificial sequence
  synthetic
  variation 11, 16, 18, 21: y=c or t
  variation (15)...(15): r=a or g
  variation (20)...(20): m=a or c
tcaccatggcytggrycycmytc

SEQ ID NO: 104 - DNA, 22 bp, artificial sequence
  synthetic
tcaccatggcctgggtctcctt

SEQ ID NO: 105 - DNA, 22 bp, artificial sequence
  synthetic
  variation (16)...(16): m=a or c
  variation (19)...(19): y=c or t
tcaccatggcctggamtcytct

SEQ ID NO: 106 - DNA, 26 bp, artificial sequence
  synthetic
tcaccatggcctgggctccactactt

SEQ ID NO: 107 - DNA, 20 bp, artificial sequence
  synthetic
tcaccatggcctggactcct

SEQ ID NO: 108 - DNA, 23 bp, artificial sequence
  synthetic
tcaccatggcctggatgatgctt

SEQ ID NO: 109 - DNA, 22 bp, artificial sequence
  synthetic
taaatatggcctgggctcctct

SEQ ID NO: 110 - DNA, 22 bp, artificial sequence
  synthetic
tcaccatgccctgggctctgct

SEQ ID NO: 111 - DNA, 22 bp, artificial sequence
  synthetic
tcaccatggccctgactcctct

SEQ ID NO: 112 - DNA, 30 bp, artificial sequence
  synthetic
cccaagcttactggatggtgggaagatgga

SEQ ID NO: 113 - DNA, 16 bp, artificial sequence
  synthetic
gtaaaacgacggccag

SEQ ID NO: 114 - DNA, 17 bp, artificial sequence
  synthetic
caggaaacagctatgac

SEQ ID NO: 115 - DNA, 440 bp, artificial sequence
  synthetic
gggcctgggctctgctgctcctcaccctcctcactcagggcacagggtcctgggcccagtctgccctgactcagcctccctccgcgtccgggtctcctggacagtcagtcaccatctcctgcactggaaccagcagtgacgttggtggttataactatgtctcctggtaccaacagcacccaggcaaagcccccaaactcatgatttatgaggtcagtaagcggccctcaggggtccctgatcgcttctctggctccaagtctggcaacacggcctccctgaccgtctctgggctccaggctgaggatgaggctgattattactgcagctcatatgcaggcagcaacaatttcgtcttcggaactgggaccaaggtcaccgtcctaggggctgatgctgcaccaactgtatccatcttcccaccatccagtaagcttggg

SEQ ID NO: 116 - DNA, 441 bp, artificial sequence
  synthetic
atggcctgggctctgctgctcctcaccctcctcactcagggcacagggtcctgggcccagtctgccctgactcagcctccctccgcgtccgggtctcctggacagtcagtcaccatctcctgcactggaaccagcagtgacgttggtggttataactatgtctcctggtaccaacagcacccaggcaaagcccccaaactcatgatttatgaggtcactaagcggccctcaggggtccctgatcgcttctctggctccaagtctggcaacacggcctccctgaccgtctctgggctccaggctgaggatgaggctgattattactgcagctcatatgcaggcagcaacaattatgtcttcggaactgggaccaaggtcaccgtcctaggggctgatgctgcaccaactgtatccatcttcccaccatccagtaagcttggg

SEQ ID NO: 117 - DNA, 441 bp, artificial sequence
  synthetic
atggcctgggctctgctgctcctcaccctcctcactcagggcacagggtcctgggcccagtctgccctgactcagcctccctccgcgtccgggtctcctggacagtcagtcaccatctcctgcactggaaccagcagtgacgttggtggttataactatgtctcctggtaccaacagcacccaggcaaagcccccaaactcatgatttatgaggtcagtaagcggccctcaggggtccctgatcgcttctctggctccaagtctggcaacacggcctccctgaccgtctctgggctccaggctgaggatgaggctgattattactgcagctcatatgcaggcagcaacaattatgtcttcggaactgggaccaaggtcaccgtcctaggggctgatgctgcaccaactgtatccatcttcccaccatccagtaagcttggg

SEQ ID NO: 118 - DNA, 438 bp, artificial sequence
  synthetic
atggcctgggctctgctcctcaccctcctcactcagggcacagggtcctgggcccagtctgccctgactcagcctccctccgcgtccgggtctcctggacagtcagtcaccatctcctgcactggaaccagcagtgacgttggtggttataactatgtctcctggtaccaacagcacccaggcaaagcccccaaactcatgatttatgaggtcagtaagcggccctcaggggtccctgatcgcttctctggctccaagtctggcaacacggcctccctgaccgtctctgggctccaggctgaggatgaggctgattattactgcagctcatatgcaggcagcaacaattatgtcttcggaactgggaccaaggtcaccgtcctaggggctgatgctgcaccaactgtatccatcttcccaccatccagtaagcttggg

SEQ ID NO: 119 - DNA, 438 bp, artificial sequence
  synthetic
atggcctgggctctgctgctcctcaccctcctcactcagggcacagggtcctgggcccagtctgccctgactcagcctccctccgcgtccgggtctcctggacagtcagtcaccatctcctgcactggaaccagcagtgacgttggtggttataactatgtctcctggtaccaacagcacccaggcaaagcccccaaactcatgatttatgaggtcagtaagcggccctcaggggtccctgatcgcttctctggctccaagtctggcaacacggcctccctgaccgtctctgggctccaggctgaggatgaggctgattattactgcagctcatatgcaggcagcaacaatgtcttcggaactgggaccaaggtcaccgtcctaggggctgatgctgcaccaactgtatccatcttcccaccatccagtaagcttggg

SEQ ID NO: 120 - DNA, 441 bp, artificial sequence
  synthetic
atggcctgggctctgctcctcctcaccctcctcactcagggcacagggtcctgggcccagtctgccctgactcagcctccctccgcgtccgggtctcctggacagtcagtcaccatctcctgcactggaaccagcagtgacgttggtggttataactatgtctcctggtaccaacagcacccaggcaaagcccccaaactcatgatttatgaggtcagtaagcggccctcaggggtccctgatcgcttctctggctccaagtctggcaacacggcctccctgaccgtctctgggctccaggctgaggatgaggctgattattactgcagctcatatgcaggcagcaacaattatgtcttcggaactgggaccaaggtcaccgtcctaggggctgatgctgcaccaactgtatccatcttcccaccatccagtaagcttggg

SEQ ID NO: 121 - DNA, 442 bp, artificial sequence
  synthetic
atggcctgggctctgctgctcctcaccctcctcactcagggcacagggtcctgggcccagtctgccctgactcagcctccctccgcgtccgggtctcctggacagtcagtcaccatctcctgcactggaaccagcagtgacgttggtggttataactatgtctcctggtaccaacagcacccaggcaaagcccccaaactcatgatttatgaggtcagtaagcggccctcaggggtccctgatcgcttctctggctccaagtctggcaacacggcctccctgaccgtctctgggctccaggctgaggatgaggctgattattactgcagctcatatgcaggcagcaacaatttatgtcttcggaactgggaccaaggtcaccgtcctaggggctgatgctgcaccaactgtatccatcttcccaccatccagtaagcttggg

SEQ ID NO: 122 - DNA, 428 bp, artificial sequence
  synthetic
ccttcattttctccacaggtctctgtgctctgcctgtgctgactcagcccccgtctgcatctgccttgctgggagcctcgatcaagctcacctgcaccctaagcagtgagcacagcacctacaccatcgaatggtatcaacagagaccagggaggtccccccagtatataatgaaggttaagagtgatggcagccacagcaagggggacgggatccccgatcgcttcatgggctccagttctggggctgaccgctacctcaccttctccaacctccagtctgacgatgaggctgagtatcactgtggagagagccacacgattgatggccaagtcggttgtgtcttcggaactgggaccaaggtcaccgtcctaggggctgatgctgcaccaactgtatccatcttcccaccatccagtaagcttggg

SEQ ID NO: 123 - DNA, 441 bp, artificial sequence
  synthetic
atgacctgctcccctctcctcctcacccttctcattcactgcacagggtcctgggcccagtctgtgttgacgcagccgccctcagtgtctgcggccccaggacagaaggtcaccatctcctgctctggaagcagctccaacattgggaataattatgtatcctggtaccagcagctcccaggaacagcccccaaactcctcatttatgacaataataagcgaccctcagggattcctgaccgattctctggctccaagtctggcacgtcagccaccctgggcatcaccggactccagactggggacgaggccgattattactgcggaacatgggatagcagcctgagtgcttatgtcttcggaactgggaccaaggtcaccgtcctaggggctgatgctgcaccaactgtatccatcttcccaccatccagtgagcagtta

SEQ ID NO: 124 - DNA, 441 bp, artificial sequence
  synthetic
atgacctgctcccctctcctcctcacccttctcattcactgcacagggtcctgggcccagtctgtgttgacgcagccgccctcagtgtctgcggccccaggacagaaggtcaccatctcctgctctggaagcagctccaacattgggaataattatgtatcctggtaccagcagctcccaggaacagcccccaaactcctcatttatgacaataataagcgaccctcagggattcctgaccgattctctggctccaagtctggcacgtcagccaccctgggcatcaccggactccagactggggacgaggccgattattactgcggaacatgggatagcagcctgagtgcggctttttttggaactgggaccaaggtcaccgtcctaggggctgatgctgcaccaactgtatccatcttcccaccatccagtgagcagtta

SEQ ID NO: 125 - DNA, 345 bp, artificial sequence
  synthetic
cccgggcagagggtcaccatctcttgttctggaagcagctccaacatcggaagtaatactgtaaactggtaccagcagctcccaggaacggcccccaaactcctcatctatagtaataatcagcggccctcaggggtccctgaccgattctctggctccaagtctggcacctcagcctccctggccatcagtgggctccagtctgaggatgaggctgattattactgtgcagcatgggatgacagcctgaatggttatgtcttcggaactgggaccaaggtcaccgtcctaggggctgatgctgcaccaactgtatccatcttcccaccatccagtgagcagtta

SEQ ID NO: 126 - DNA, 432 bp, artificial sequence
  synthetic
atggcctggacccctctcctgctccccctcctcactttctgcacagtctctgaggcctcctatgagctgacacagccaccctcggtgtcagtgtccccaggacaaacggccaggatcacctgctctggagatgcattgccaaaaaaatatgcttattggtaccagcagaagtcaggccaggcccctgtgctggtcatctatgaggacagcaaacgaccctccgggatccctgagagattctctggctccagctcagggacaatggccaccttgactatcagtggggcccaggtggaggatgaagctgactactactgttactcaacagactacagtggtaatcatgtcttcggaactgggaccaaggtcaccgtcctaggggctgatgctgcaccaactgtatccatcttcccaccatccagtgagcagtta

SEQ ID NO: 127 - DNA, 426 bp, artificial sequence
  synthetic
atggcctggactcctctctttctgttcctcctcacttgctgcccagggtccaattcccaggctgtggtgactcaggagccctcactgactgtgtccccaggagggacagtcactctcacctgtggctccagcactggagctgtcaccagtggtcattatccctactggttccagcagaagcctggccaagcccccaggacactgatttatgatacaagcaacaaacactcctggacacctgcccggttctcaggctccctccttgggggcaaagctgccctgaccctttcgggtgcgcagcctgaggatgaggctgagtattactgcttgctctcctatagtggtgcttatgtcttcggaactgggaccaaggtcaccgtcctaggggctgatgctgcaccaactgtatccatcttcccaccatcc

SEQ ID NO: 128 - DNA, 331 bp, artificial sequence
  synthetic
agtggtcctgggacagacggccaggattacctgtgggggaaacaacattggaagtaaaaatgtgcactggtaccagcagaagccaggccaggcccctgtgctggtcatctatagggataacaaccggccctctgggatccctgagcgattctctggctccaactcggggaacacggccaccctgaccatcagcagagcccaagccggggatgaggctgactattactgtcaggtgtgggacagcagcacttatgtcttcggaactgggaccaaggtcaccgtcctaggggctgatgctgcaccaactgtatccatcttcccaccatccagt

SEQ ID NO: 129 - DNA, 417 bp, artificial sequence
  synthetic
actcctctcctcctcctgttcctctctcactgcacaggttccctctcgcaggctgtgctgactcagccgtcttccctctctgcatctcctggagcatcagccagtctcacctgcaccttgcgcagtggcatcaatgttggtacctacaggatatactggtaccagcagaagccagggagtcctccccagtatctcctgaggtacaaatcagactcagataagcagcagggctctggagtccccagccgcttctctggatccaaagatgcttcggccaatgcagggattttactcatctctgggctccagtctgaggatgaggctgactattactgtatgatttggcacagcagcgcttatgtcttcggaactgggaccaaggtcaccgtcctaggggctgatgctgcaccaactgta

SEQ ID NO: 130 - DNA, 393 bp, artificial sequence
  synthetic
tttctgttcctcctcacttgctgcccagggtccaattctcagactgtggtgactcaggagccctcactgactgtgtccccaggagggacagtcactctcacctgtgcttccagcactggagcagtcaccagtggttactatccaaactggttccagcagaaacctggacaagcacccagggcactgatttatagtacaagcaacaaacgctcctggacccctgcccggttctcaggctccctccttgggggcaaagctgccctgacactgtcaggtgtgcagcctgaggacgaggctgagtattactgcctgctctactatggtggtgcttatgtcttcggaactgggaccaaggtcaccgtcctaggggctgatgctgcaccaactgtatcc

SEQ ID NO: 131 - DNA, 417 bp, artificial sequence
  synthetic
atggcctgggctctgctgctcctcactctcctcactcaggacacagggtcctgggcccagtctgccctgactcagcctgcctccgtgtctgggtctcctggacagtcgatcaccatctcctgcactggaaccagcagtgatgttgggagttataaccttgtctcctggtaccaacagcacccaggcaaagcccccaaactcatgatttatgagggcagtaagcggccctcaggggtttctaatcgcttctctggctccaagtctggcaacacggcctccctgacaatctctgggctccaggctgaggacgaggctgattattactgctgctcatatgcaggtagtagcacttatgtcttcggaactgggaccaaggtcaccgtcctaggggctgatgctgcaccaactgtatccatc

SEQ ID NO: 132 - DNA, 348 bp, artificial sequence
  synthetic
cagtctgccctgactcagcctgcctccgtgtctgggtctcctggacagtcgatcaccatctcctgcactggaaccagcagtgacgttggtggttataactatgtctcctggtaccaacagcacccaggcaaagcccccaaactcatgatttatgaggtcagtaatcggccctcaggggtttctaatcgcttctctggctccaagtctggcaacacggcctccctgaccatctctgggctccaggctgaggacgaggctgattattactgcagctcatatacaagcagcagcacttatgtcttcggaactgggaccaaggtcaccggcctgggggctgatgctgcacca

SEQ ID NO: 133 - DNA, 20 bp, Artificial Sequence
  synthetic
aacaaccgagctccaggtgt

SEQ ID NO: 134 - DNA, 19 bp, Artificial Sequence
  synthetic
agggcagccttgtctccaa

SEQ ID NO: 135 - DNA, 20 bp, Artificial Sequence
  synthetic
cctgccagattctcaggctc

SEQ ID NO: 136 - DNA, 20 bp, Artificial Sequence
  synthetic
catcacaggggcacagactg

SEQ ID NO: 137 - DNA, 19 bp, Artificial Sequence
  synthetic
gatttgctgagggcagggt

SEQ ID NO: 138 - DNA, 21 bp, Artificial Sequence
  synthetic
ccccaagtctgatccttcctt

SEQ ID NO: 139 - DNA, 20 bp, Artificial Sequence
  synthetic
gctgaccaacgatcgcctaa

SEQ ID NO: 140 - DNA, 19 bp, Artificial Sequence
  synthetic
taagcgccacactgcacct

SEQ ID NO: 141 - DNA, 24 bp, Artificial Sequence
  synthetic
cctgccagattctcaggctccctg

SEQ ID NO: 142 - DNA, 23 bp, Artificial Sequence
  synthetic
ctgattggagacaaggctgccct

SEQ ID NO: 143 - DNA, 30 bp, Artificial Sequence
  synthetic
ccttcatactcttgcatcctcccttctcca

SEQ ID NO: 144 - DNA, 35 bp, Artificial Sequence
  synthetic
ttccttctcttctgtgactcaattatttgtggaca

SEQ ID NO: 145 - DNA, 159 bp, Artificial Sequence
  synthetic
tctggcacctcagcctccctggccatcactgggctccaggctgaggatgaggctgattattactgccagtcctatgacagcagcctgagtggttctgtgttcggaggaggcacccggctgaccgccctcggggctgatgctgcaccaactgtatccatc

SEQ ID NO: 146 - DNA, 159 bp, Artificial Sequence
  synthetic
tctggcacctcagcctccctggccatcactgggctccaggctgaggatgaggctgattattactgccagtcctatgacagcagcctgagtggttatgtcttcggaactgggaccaaggtcaccgtcctaggggctgatgctgcaccaactgtatccatc

SEQ ID NO: 147 - DNA, 159 bp, Artificial Sequence
  synthetic
tctggcacctcagcctccctggccatcagtgggctccagtctgaggatgaggctgattattactgtgcagcatgggatgacagcctgaatggtgctgtgttcggaggaggcacccagctgaccgccctcggggctgatgctgcaccaactgtatccatc

SEQ ID NO: 148 - DNA, 159 bp, Artificial Sequence
  synthetic
tctggcacctcagcctccctggccatcagtgggctccggtccgaggatgaggctgattattactgtgcagcatgggatgacagcctgagtggtcgggtgttcggcggagggaccaagctgaccgtcctaggggctgatgctgcaccaactgtatccatc

SEQ ID NO: 149 - DNA, 153 bp, Artificial Sequence
  synthetic
tcggggaacacggccaccctgaccatcagcagagcccaagccggggatgaggctgactattactgtcaggtgtgggacagcagcactgctgtgttcggaggaggcacccagctgaccgccctcggggctgatgctgcaccaactgtatccatc

SEQ ID NO: 150 - DNA, 156 bp, Artificial Sequence
  synthetic
tcagggacaatggccaccttgactatcagtggggcccaggtggaggatgaagctgactactactgttactcaacagacagcagtggtaatgctgtgttcggaggaggcacccagctgaccgccctcggggctgatgctgcaccaactgtatccatc

SEQ ID NO: 151 - DNA, 159 bp, Artificial Sequence
  synthetic
tcagggacaatggccaccttgactatcagtggggcccaggtggaggatgaagctgactactactgttactcaacagacagcagtggtaatcatagggtgttcggcggagggaccaagctgaccgtcctaggggctgatgctgcaccaactgtatccatc

SEQ ID NO: 152 - DNA, 159 bp, Artificial Sequence; identical to SEQ ID NO: 146
  synthetic

SEQ ID NO: 153 - DNA, 159 bp, Artificial Sequence
  synthetic
gatgcttcggccaatgcagggattttactcatctctgggctccagtctgaggatgaggctgactattactgtatgatttggcacagcagcgctgtggtattcggcggagggaccaagctgaccgtcctaggggctgatgctgcaccaactgtatccatc

SEQ ID NO: 154 - DNA, 153 bp, Artificial Sequence
  synthetic
cttgggggcaaagctgccctgacactgtcaggtgtgcagcctgaggacgaggctgagtattactgcctgctctactatggtggtgctcgggtgttcggcggagggaccaagctgaccgtcctaggggctgatgctgcaccaactgtatccatc

SEQ ID NO: 155 - DNA, 153 bp, Artificial Sequence
  synthetic
cttgggggcaaagctgccctgaccctttcgggtgcgcagcctgaggatgaggctgagtattactgcttgctctcctatagtggtgctcgagtattcggcggagggaccaagctgaccgtcctaggggctgatgctgcaccaactgtatccatc

SEQ ID NO: 156 - DNA, 165 bp, Artificial Sequence
  synthetic
tcaggcctgaatcggtacctgaccatcaagaacatccaggaagaggatgagagtgactaccactgtggggcagaccatggcagtgggagcaacttcgtgtctgtgttcggaggaggcacccagctgaccgccctcggggctgatgctgcaccaactgtatccatc

SEQ ID NO: 157 - DNA, 164 bp, Artificial Sequence
  synthetic
tctggcacgtcagccaccctgggcatcaccggactccagactggggacgaggccgattattactgcggaacatgggatagcagcctgagtgctggccccgggtgttcggcggagggaccaagctgaccgtcctaggggctgatgctgcaccaactgtatccatc

SEQ ID NO: 158 - DNA, 22800 bp, Artificial Sequence
  synthetic
aagctctaaaactacaaactgctgaaagatctaatgactaggacagcctagtaattttcataggggcataaatgtgaaacgccttgtgcatcgtagaagaaagcagaagagaaagcattcccaatttcttaactgccttttacctatattaatcagtaatatactggcttttacctctgttaatcataataaacaaattctcaataaattttatcgatactcttcaatgcctgctcagcaacattttccgaaggcagctcaagatattaaataactcataagggccaacctcctattgcagcattctttgggatttaaccagtttcccaagactcttttcacaatgttaagatgttagaaatagatccaaaactaggtgatatatcccctagtaaaactgtgaggtcaaacttgtctggctaatgcttccatttaaaaatttctctttcttgatccttcattgtatgtacacaataaatcaggggaaaactttaactgagtgaatcaaagtattctcattattataataggagcttcacacacacacaaaaaaatcaattctattactctcagcctcagttcctaaagccaagttaaagtcctgttctaagatcattgttgcatgaccatatgtattccaggtctaatctaaactgtggataaatcccagcaggacattagagatttttgtgagagtaagcatataggattcagggtttatgagctttagatttttcttgtcaaaatgaatgagagttgccatatctaaaaattattcccagataaataaaattcactacctagaattaatttatgcatataagtagaaatgctatctccctttttaccatccaaagtggaaagcctcatggaactagaaattaatattagaaaaatcagttaataaaagtatgtcatttcatcaattcaataagttataatagcaaaaaaccataataaattatcacttaaatgtcaatacatttataaactatggtacataaataggatattgaatagccattgatgctcctgatgaaaattagcaggcagtgataaatgataaatatgaagcacatgtcaataaataaaataagttttatgtaatttaggagaaaatggtgataatgacacaaaatgtgaattatggatgcatctataaaattctttgtacatttgtgaattgtaaatatttatcttagagacattattactttgtatatgttccatttgctcacctatatgtcccagtctccttacaaatgctatggccaaagaaataggcatacatacatcctttgcaggctgaggcaggaaaaagatcttacggaattttccagtctatcctttatctgtataagcaacttaagaggccatgtgctccaaatggtgcaaatacaagatggtagagcctctgtctgcctggatccttgagtggctgcatggagcagagcacctttctggccctggtgaagattgtagcatgagcaagatataagcatttgttggagctaggccatgagatttggggcagtggtataacctaccctattatggaaaatataaatacacaaaacagaaaagagagagagaagtgagagaagactgtgagagaagtgcatgagagaagactgtgttttgttcatttcctataatcctatatcaccatgggatcctgtgccttctggtgatcaaactaatgttctacagctccaaagaagaatgctcgcctaacgtctccattccaatgacctagagactaaaagccaaaaagaaccttagaaattatctattgcattctttgatgtaaggaaatatcttagagggcacagatagaaatatcttaacccaggtcacttagttcgtggcagagctgaggctaaaaccaggccttttgactcctaattttgtgctctttacaccttctcacatcacttctccaacccaaagtctagcagaaaaggctaaaataagatatatgcatagatttgctattataagtccatgtacttcctcagacgctttaagatggggcttctcatggttcacaataagcagcagagggaagtgaataactatcttcgtctcccctactgctatttgtgcagtttgaagcttatctcttaaatcatgttttcttctcgtagtaaatactacaacttgtgccttttatgtgtgtataaattttaatataatttttttccatgaaccattcaagtaaaatggacactccaaaaagatgttcaataaggttacatggcttcacattgccccctctacaccatcttgtggagctacacattcacctcacccaaatttgagaaaaataatcaagaaaatgactctcactagcagtgagaccaagtccataagcactaatgtcatcagtgcacactgcagcctcatgctgccaagcatgttttgggcgtatccctggactggtttggtgacatgatcaaaggtacattttccacctgcatagccccatcctggatctatagccttccttgtgtctttgtgaacaacctagtgtgaactcaaagtatgagacagatctcaattaatttagaaagtttattttcccaagattaaggacaagcccatgataaagcctccagaggtcctgatatatgtgcccaagggggtcggggcacagcttggtgttatacattttagggagacaagaaacatcaatcgatatgtagaagatgtgcatcgctttggtctggaaaggtgtgacaactcaaggcagggaagggggcttcctgctggggttgcattgttttgagtctctgatcagcctttcacatgtgaaaggcaggtagagaaatagtcatttatgccttagtctggcttattgaaacagtagggcagaagaagcattgcatatgcatttgtctgaagtgaacagagggatgactttgagctctgtcctttctttgtccacaaggaattaccttgtgggcaaattgtgagggaggtatgtagcttttttttctttgtagctatcttatttaggaataaaatgggaggcaggtttgcctgatgcaattcccagcttgactttcccttttggcttagtgatttttggggtcctgaggtttattttttctttcacattagtataactacttttctttttctaattccttttctacttgtatgtgttacagctgacttatgttacttgcaaaaagaattctgactaatgcaccatctgactagaaggcagggttcttcgatgataacgaatcctccagaatctagtaaacagaattgcctgaaaaagaggtgggtgtcttcttggggaatttctcatggcaatgaatggcaactggccaaaggatttatgaccagactgagctctcttttatctattctgttactcaccaagacctattagggtttgtgctccacagggacactggtttctaagttctagggttaaacagtccactcccaggcccaccacaccataccctcctgacatctggtgaacagcaataaaattgtttcttattctgaaaatcctccaatacttccaccatccccaaaaatgcagtggaggaggagagaaaatgaattgttccattagagaacacaatatccattatattattcttggcctttgagataccttacaaaacaaatacaaaaaaagtcccaatttaacatcttttaataatctttacaaaacagaacacatctcctttcttgataatagtcaagaggctcagtggcaactgtggtgaaaagtgtcagattctggtcatgtttcaaaggtagaaaaaatagaatttgttaacatattggatgtgaggcgtgggagaaacgtgaaatcaaggtggttgcaagtgtttaacctgagcaactagagaatttggaaggacattttctgagatggggaaggcaggcgggaatcagggattagagttgaacatattagacatttgagatgcctgctagacctctaattggcaatatcccttggacaggtggatgaatatgcgtgattctggagttcgggaaatagtccgggtggagatgcaaatttgggaaacagggcgaggttactagcaatgagttaaatcaatgaaggcaggctgggacctggcaggtaacccaacaagtagaggtcgaagagatgagaagaaaacagcacaggagacttagaagcagtggtcaggaggaaggagttgaaccaagaaagtgatgtcccagagccaacaaaataaggatttcttttctgtttacaaatgtaaaattaaaaggtttaataaaaagaaaatttacttttatggttggttgttattaagtggtccaaacactgtctcctatttgtagaatcagaactctctcatggcagtagaaaatttggaaagttactttttaaaaggtgtgtgcactgctgccctttgctggtcaagtttatgcactgcaaattccaaggacgattgctcgtcagcttttctcctttaaaatagctcaggctgtacaagctagaaagaacctcgcaagatattccttccaacatttgcatttgacttatgggaagtgcaggttcagccagaaaagttgtgtgcaaggccgtttatgtaagtttatcagacctgattcttacggctcttcccattgtttcgagcctcccttccattcacttcccgctcatacgcgaccaagtataggacaggagtagttattctgcactttatagcagctccactgtctggcactctgatgttctttaattacaagctttatgacagtgattctcaacctgctccactgcctccacctagtggcagaaagaagaaaatgtgtgtaactcgggagtctctggtctgaaagctccggggtatcatttcttcaaagtcttgagcttgtttttgtttgtatttatttatttatttgttttagagacaaggtctcgcactgcactccagcctgggagacagagcgagacaattcaggatctatctagtgaataaagagatatcagtaatgactgttttatattgtggctgtagcgcattcgagggataattcgattctgttctgctttcgaatgcatggctcactgtaacctccaactcccgggctcaagcgatcctcctacctcagcttctccagtagttgagcttgatttattttaaagtttcataaaattttggcatttctttccacaatatggccatgtgtgctttactataaaatattttcatcacaaaatttacatcgctggaaatccccataagccagtttgagaaacacaacccaagaaagcagaacagactcaaattatcccttaaatcccccttaaccacaaatataaaacagtccgtgactgggcgtgttggcttacacctgtaatcccagcactttgggaggccaaggcgggtggattacttgagctcaggagttcaagaccagcctggccaacatggtgaaaccccgtccctattaaaaatacaaaattattcaggagttgtggcaggcagttgtaatcccagctacttgggaggctgaggcaggagaatcacttgaacccaggaggtggaggttgtagtgagccaagattgtgccagtgcactccagcctgggcaacagagcgagacttccatcttaaaaaaaaaaaattaagtaaataaaatataaaaaaataaagcagtccctattgatatctctttattcactaaatcaacctggaattgacctgaattctgatttttttttcatcatggattttttgcattaattttgattgtttaaatattgcattaaaatattatttatcttgactactgagtttgcgggacctccttaaaatttatgaccaaggcaatgcctcactcactcgccttaccataatctgggccacatatcaggggctccaatagcaagcaacatgacttttgaacagctaagacttctctcttcactgtgaagaccagatgggccctgcaaacagtgtaacctctacatgaaaatgcacgagattccaactacaaccaggcacaaaagactctgatggtgaagtcccagccctccaagtcccaacttcctgaagggaaagagcaccccaagttctgaccagaggccagagtcataacgaagatggaatgtgagcttgacatagaaggggtggtagcacctggctcagtaatgaagaggctttcggtcctgaaggaagagctcagcacattcaaagattagaagggaggtcccagtcataggagcagggaaggagagaaggcccaataagaaacacagacaggagggaggggtcagggcaagatcatactggaaacaactagagagctaataaaagtcacagtgcccagtccccacatggaccagactcttcggaatctctaggcatcaatttgggcaccagtagttttcaaagttctccagaagattctatgcacaccagccaagggtgggaaccacaggtgttggcctagggatcatgacaatgagtttctaagtgcaataagaaacctccagagagtttaagcaggggaataatttgatttgtttcttgtttgtgatttttaaagatcagtctggttactgtgtgtaagacaataatccagaaaatctgttgctcatgaaccacatatctgtaaatttgcttcccctgtaactggatctaaccaacaaaaattagtacttactaagaaattacatgcccagggactatgctaagtaattcataaacactattttatttactcctcacagcaagtttataagagaaacgttattatttccacatttcggatgagaaatttgaggcttggggaaagttaagtaatttacctaatgtcacacccagttcataagatgcagagttaagattctaattctgtgtctaagttgatgctccatcaaacacaccacgcctccaactaggaagcaacatgctggccagaggatgctgtcatcaagtttacagaatggttagatttctaggcacagatgaataaatcaacatgttggtttgcaatagaatgaatctatccagctctgaatttgcatccaagggtttgtgagcacacaagtctaaaagtgtggcctcagctctgctaacttcatcaaggtgaatacctaggaggccaccctctgagaccaccagatggacagtccaccatctgtttacagatggtaaagccacataccagctttgccatctgatgttctctattcacattcaacatttatacaagaaatagtcatatggatccttttcaatagacagtactggggaaattgaattgccatatgcagaagaatggaactagacctctatctctcaccaaatacaaaagttaactcaagacagattaaagacttacatataagacctgtaactacaaaaacactagaagaaaacctagggaaaatgcttctggaattaatctaggtgaagaactcaggactaagatatcaaaagcacaagcaccaaaacaaaaatagacaaacaggacttaattaaactagaacgcttctgaacagcaagagaaataatcaatagagtgaacagataatctgcagaatgggtgaaaatatttgcaaactatgcatcctacagggaaataatgtccagaatttagaaggaactcaaacaattcaacaacaacagcaaaataaccccaccaaaaaagtgggcaaaggacatgaatagacatttttcaaaagaaggtatatgatatggtttggctctgtgtctccacccagatctcaccttaaattgtaataatccccacatatcatgggagagacccggtgggaggtaattgaatcatgggggcaggtttgtcccatgctgttctcatgatactgaataagtcctatgagatctgatgattttataaaggggagttcccctgcacacactctcttgcctgcctccatgtaatatgtgcctttgcttctcctttgccttctgccatgattgtgaggcctctccagccatatggaactgagtcaattaaaccactttttctttgtaaattacccaatcttgggtatgtctttattagcagcataagaacagactaatacagtgtacaaatggccaagaagcgtacaaaaaacaaaatgctcaaatcactaatcactagagaatcgcaagttaaaaccacaatgagatattatcttacagcagtcagaatgcctattattaaaacaccaaaaaataacatgttggcaaggatgcagagaaaagggaatacttacacattattagtgggaatgtaaactagtacagcttctgtggaaaacactatggagatttctcaaagaactagaaatagaactaccatgtggttcagcaataccacaactgggtatctacccaaagggaaataaattattatataaaaaagatatctgcactcacttgtttattgcagcactattcacaatagcaaagatatggaatcaacccaagtgtccatcaacagatgattggataaagaaaacgtggtgtgtgtgtgtgtgtgtgtgtgtgtgtatacacataccacaatgaaatactattcagctataaagaaaagaatgaaatcatgtcttttgcagcaatgtggttggaactggaggccattatcttaagtggataattcaaaaacagaaggtcaaatgtcacatgttctcacttataagtgggagctaaatgatgtgtacacatggacatagagtgtggtatgataaacactggagattgagatgggtggaagggtggaaggaggttgagtgatgagaaaatactaaatggatacaatatacatgattcaggcgatagatacactaaaagcccagacttcaccactacacagtatagctatgtagcaaaattgcacctgtattgcttaaatttatacaagtaaaaaaaagatcgtacgaattctgttttttattctctatgaaattactactgagagtattatccaatgccgtttctatgcagtgcccccaatattatccatttagcagctcctatgcaatgccccaagatagaaattgtcttcaacttttatcccaggaaaaccttcagtcacacgtagaaactagaaatttttcccctagatgaaagttatgtaacataacacattatcttcatttagtcggtttccaagaagctcagaaccagattttatgttcaatcaaaaactgcttattttaagtgaggtttactgaggtataaattacaataaaagccaccttttcgtgtatatttctataagttttggcaaatgcatagctgtgtaaccacaaccacattcaagatataggacaagtccctcatcctttaaagttcctttatgccccttccttcaccccagcccttggcaaccactggtttttgtctgatccaatcgtttgcctcttcctgaatgtcatgtaaatagagccatgcaatgtgaagccttttgagtctggctttgttcacttgttcacttaggagaatgcatttgagattcatctttgctgtttcgtgtagcactagttcactgtctattgttgagtagtattccattgtgtggatatgccacagattgtttatctagttaacaatttaaagccatttggtcatttctaatttttagctgctaagaataaagttgctgtaagctttccaatgcaggtttttgtgtgaactcaggatttcatttcgcttgggtaaattcctagctttgggactgctgagtcatctggtaggtgtatgttgaactttataagaaactgccaaactgttttccaaagttgctgtgctcttttgcactcccatcagcagtgaatgagggttccacttgctcgagcctagtattttaacttcactatataccttctttgatgacatatcctttcaaatttttggtcaagtttttattggggtgttgttactatggactgtgagagttctttgtatattctgcatatgatttttttctcacatttgtgttttatgaatatgttctcccaatgtgtggcgccttttattttcttaacgtgccatgtgaagagcagaagtttaattttatgatgtccaaattatctttttttcttttcttttttagatcaaaataggggtctattttgattaccactgttattttatctccatttgattttcgatttttatttttatttttctaatttcattgtaaatttttaattaaacccaaatattctaggggaaagaggcaagataaaaatagtctaacttgggcataaattttagagtcatattctcttgccgagaaaggaaactagctctcttacattgattgtttaatttcagacgtcactactttatgaggatgcccaaattatgggctttaaaaaatatatatccaaacaggggttcagaaagaataactaatttgtccacaacaacacaaaaaatgattccaccataagtttgcccagtgacagggtctatattattttctatatatcaaattctacaactggttcttaaagctactgtacataacctaagttaaaatattaggtattagttgataagacattttatcatctatgaaatgttgcctgttgtcatagttagagaatcttttaaaatatggagctattttcatagattaaactatgccagttaaaagttgggtaaaaagaactacagaataatatttatgtttatcgtgtaaggttttaaagcaaactccaagtcattttcatcaatgaaatcaataaggttttgcaaatatatatgtatgaaaatactgatttaaaatgcaaataaggggagagtttgagagagagagagagaccaaatgattttataattctagtaagtttataggtttatggggtttttacgtacttttctacccaacttgtctataagactttaatgaatcacttagaatttttaaaataatttattattactctgtacctgttctttactctgcaaatcttaccttgcccttttgtctaaaagcaataaaatctgacctggtttatatcgtatcattgattttgttacttagcaagcacagtgatccattaggcctatgtaggctcatggtttatacaacactgccatctgctgacagagtgtgacagtcacagtcagcaacacgagaccactttattttcatttttagtgtttatagaaatatgaatatacacaaatagtataatgaaccctaagcttcacaaattaacattttgctaatcttgtttcaactaccgcctcccccctcatccaattactctgttctctcacctcctcacacacagacactggcagtatttttcagccaatcattaatacgttgccaactgataaggacttttaaaaaacaaccaccattccattatgattcccagcataattgagagtaattccctaatatccaatacccattttctattccaatttccttgattgtctttaaactgtttttaccctaagtttgcttaaatcaaagtccaggtcctgttaaacatatggttaagttttacccaaacccaaataaataaataaataaataaataaataacctattttttccaattccagggaatagtgaaagagggtaaatgccattatttagaaacataaatcacatcataggactagaattatcttgaagtcaaaattgaagactgaaaatggaaaagaaaggtatagactaaacttatttaaaaacttcaatgcagaactctaagagaagatattagaaagttgtaccagcattcattattcagtattcatcagtattcactcagctatatgtagttgaaatctaactagaggagcttgatcagataaagagatacatttttctcaccaaggcggactctggaggcaggtggttcagagctagacagctgctgcaggacccaggtcctttccctgcctgctcctccactctagcttgtgactttcatcctgcaagatgggtgtttctgccaagttccagatagaagaagatagaacacaaaggagaaataagcagtggtgcctctgtccatcaagcaaaatttttccagaaatgcacaatagatttcagatgatgtctcaacagtcctaactgcaaagaagctgaggaattagatttttggctgggacactgttgccctgtaaaaaaattgggattctgttattaaagaataagaggagggaagaaagattgaaaactcctatgcaatagtgaaaaaaataagaaactcaataaaaaagtgggcataccttaaaaacaggcaattcacaacagatgagaccccaatagccaataaacatttttaaatggtcaacctcatgagtgatcagaaaacacaaatatgtattttaaaccaaaaataaaatacaatgtattgaccatttgagtggaaaaaaattaaaaagcctgataatatcaagtattggagaggatgtagagtgaggaaactccatggaggacctatcattgcaaatgtgggaatgaaacttaatacacgaatttgaggccaatttgtaaattgaaaaatgcgcacaccctgcaaccaagtaccccttgcaatatttttgaaaagacaaaaacgttatgtaaatggaatcatgcaatatgtgacctttatactcagcataatgcccctcagatccattgaagtcatgtgtatcaacagctcactattttttttttaattttttttagagacagagtctcactctgtcacacagggtggagtgcagtggcgagatcataactctctctagcagcctcgaactcctgggctcaagcatcctcctgcctcagcctcccaagtagctaggactacaggcatgggacacaacacacagctaatttttttaaattttttttagagacatggtctcactatgttgcctacgctggtctcaaactcctaggtcaagcgattctcccacctctacttcacaaagtgctgtaggtatgtaggtatggattgtaggtatgaaccaccgtgcccaactcactactttttattactaattattccatgggatggatgtaccgcagtttgttttaccattaatctattgtaggacattttgactgattccagtttttttttaatacaaataaaaccactatgaatagttgtgtattgtatacgtttttgtgctaagttttcatttttctgggataagttttcatttctttgggcttttactgtatccttgatattataatatgttacatcttcagttttattctattcaatatataatcttttattttccttgaaatctcccatggattgtttagaagtgtgttgttttgtttccaagggtttggcatttttcccattatttttctattatcgatttccagtttgattccaggtggtcagagaacacacttcatgtgatttcagttctattaaatttgttgaggtttgttacatggcccagtatatggcaattttggtatatgttccatgagcacttgaaaagaatgcgaattctgctggtgctggttggagttttccagcaatgttgatttatgatcttactcattgatggtggtgttgagtttgatgtgttcttacgatggcagctttaacattcttgtcaggtaattctaacgtctctgtcatgtcagtattagcgcctcttaactgtctcatcaaagctgagattttcctggttcccctggttcctgttgggatgtgtggttttcatttgaaatctggactttggagtattgtgttatgaggctttggatctcatttaaactcatctcagcgaatttcctctcttgccactcaggaaggagaagttgggtgtttgaatggagcagagccgttactgcctaagaattgttttactgggcttcccctttctttctcctttgactagagagagccagctttttattagggctttatgtttttctgggcctgttggtgtttctgggttgacaaacttctccagaaccaagtctggaatggatgaggcaaaaagaaaccccgtggaatgcactgctgggtcgctccttgggtcccaatgttcctaactggtctgccttcttctctccagcttccagagtcttcataagtttgctttacgtacaatgtccggggtttttactttacttgagagaaataggtaaaagtaattctactccatctttcaggaagcaaaagcccccttgtgtatttttttaaactttcaaaaacaaaacaaaaggcagctgcaacagtaaagaagctagtaacacccttggtgggaaattcaagtccaaatacacattttaagtttggctagccagtgagaacatcagaatagttcaggttttaaacaaatttatatttatgattatgcatatactaaaagctgaaggcatcttatatttactaagcacctattttgttcttgttaaaaagacagaattccattccctaggaaatttgacctggcagctggagctgatccacctggccactagagcacagagcagggagagtagtagccctgccccagccacccctcaagacaggattctttctctgggaactgtaggtaacactaaatcgttctggaacacaacaacgaaagaagaaaggaaagagaaagaaagaaaggaagaaagagagagagaaggaaggaagggagggagggaaggaaggaaggggaagggaagggaatggaagggaaggaaggaaggaaaaggaaggaagggagggagagagggaggaaggaaggaaaggaaaggaaggaaggaagaaggaaagaaaaaaagaaagaaagaagaaagaaagaaagacaagaaagaaagaaagaaagaaagaaaggggaaagaaaagaaagaggaaagaaagagaaagaaagaaaagaaagaaaggaaagaaagagaaagaaagaaaaagaaagagaaagaaagagaaagacaagaaagaaaaaggaaagaaaagaaagagaaagaaaagaaagaaaggaaagaaagagaaagaaagaaaaagaaagaaagaaaagaagaaagagaaagaaagaaagaaaaagaaagaaagaaagaaagaaagaaaaagaaaaagaaaggagaaaatgacagcaattacttttgcaacaacctaatataagttttttaaaagttaaatattctgttccatgcattgctggataccttataaataacagggcatcctatgacctgaatttcccaaattatgagttgagggtttgaactagttttaaaaaacaaggaggccaggcgcactggctcatgcctgtaatcccagcactttgggaggctgaggcaggtggatcacgaggtcaggagctcgagaccagccttaccaacatagtgaaacaccgcctctactaaaaatacaaaaattagccgggcgtgatggtgcgcacctgtaatctcagctactcagcaggctgaggcaggagaatcgcttgaacccagaaggcggaggttgcagtgagccaagatcacagcattgcactccagcctgggcgacagagggagactccgtcttcaaaaaaaaaaaaaaagacaaggaatctgtaaaacaggcactggaagtatatgcacttttattttcattctatgctatccgatgcctactgctatttcccttcatatttaacctccaacagctgcattttgctccctccagaccacctgattggagctcacgtgctcccacacagtacctccaaccagagagagtcgagtcccacagaaaggcgtaacaatcaccagtaattttgcacttattttacattgtgccttgatacagagtactcaatgaatgctctttgaatcatatttaataaatatgtgtatttgggattgtagcatattgcagctacctggatatataatttaattagaaaaaaaattttgtgtggctcaatcaacaaacgacttttctctctctctctttctctttctccctctctctctctttcttctcagttgatgttgctggagttcagtgttgtgcagatggcagtgacaaatgccatgggcacatgagatatgataaaaggtccctgaagaaggtggagaaccagttatcttatgaaattttccagagtgggtactggatctctcctgtctggcaccatgctggcctcagcccaaggggaatttccttccagagacagagggcagtgattgaggtggggagacagatcgtaacactgagacttacatgaggacaccaaacagaaaaaaggtggcaagtatagaaaattctttcttctggacagtcttctctgttctaacttcagcaaaattctccccccagtggatgctattgcacaaccctacatatgctatgttttttcctatacacacttacctatgataaaatgcattaattagtcacagtaagaggttaacaacaataactagtaataaaatagaacaattcagtaaaataagagttacttgagcacaaacactaggatatcatgacagtcaatctgatgaccaagagggctactaagcatctaaacaggagggtaagtgtagacagcatggagacgctggacaaagggatgattcagtcccaggctggtatggagcggaagggcatgatatgtcatcacgctactaaggcacacaatttaaaatgagtaaattcttatttctagaaatttctttttaatattttcagactacagttgcctacaggtaactgaaaccccagaaagcaaaattgttgataaggaggtactactgtacatcgtcctttgaaccaactttatcatttgctagtatatacatatatacctacatacatacatatacacatacctgcacacacctatatgtatacgtacacacacacacacgcacacacacacactcacatctactaatgttagaataagtttgctaaataagatgcacaacttgttaatgtcctacagagcaataaaaccataagcattggggttatcttttctactagataaaaatccattatcattttcataaagttttctttacattaacatctaacttttgcaatctagtttttaatcatcataaataggaagcaaatgaactgtttctctagtgaatcaaatatccttgaaaacatacatagtcatctttttggtttatttttatttttagataaattatttaaagttttaaataatttaacattcacaatagtttgtgactgtatattttgacttggtccttcaaacttaatttgtacttttatgtatcgtgcttacctcaattttttattcacttttcctaaactttgctggattggtttattatttttgtctatttcttttccttctagtggtttgggagggttttttaaatcccattactattgaatgcctattaacttgccccctttttctttcaatctctattcccacggcctgaagcatgagggccaagctgtctgtaaccagcagagagatgacccaggtgttattccactctccactgtccacctatcaccattcccagcccgatagctctgaagtacggcttttctggggctctgtggggaaaactagaactggctgcttcaaggacacctcctgtttttgcaatggaaaaaatgtttctaaattccagtttctctatgaattcaatgacatggtttaaatctctgtggtgttcttcaaagttttttcttctaataggacctctcatgattctccaaccacgaaataaattcattatcatttttatatttcttctgtcattgcaaaggaggttttgaaagagtggaggacgcgctaatgaactcaaaaatccacactattccttgtttccatctgttgttcattcattgtttccattggcctgtccgcctcctatcctccttcttagacttggagctctagcctcagccaggatagggaaaagagagatcagactgttactttgtctatgtagaaaaggaagacataagaaactccattttgatctgtatcctgaacaattgttttgccttgagatgctgttaatctgtaactttagccccaaccttgtgctcacagaaacatgtgttgtatggaatcaagatttaagggatctagggctgtgcagaatgtgccttgttaacaacatgtttacaggcagtatgcttggtaaaagtcatcgccattctccattctcgattaactaggggcacagtgcactgcggaaagccgcagggacctctgcccaggaaaactgggtattgtccaaggtttctccccactgagacagcctgagatatggccttgcgggatgggaaagatctgaccgtcccccagcctgacacccgtgaagggtctgcgctgaggaggattagtaaaagaggaaggcctcttgcggttgagataagaggaagccctctgtctcctgcatgcccctgggaacggcatgtctcagtgtaaaacctgattgtacattcgttctattctgagataggagaaaaccgctctgtggctggaggcgagatatgctggcggcaatgctgctctgttgttctttactacactgagatgtttgggtgagagaagcataaatctggcctacgtgcacatccaggcatagtaccttcccttgaatttacttgtgacacagattcctttgctcacatgttttcttgctgaccttctccccactatcaccctgttctcctgccgcattccccttgctgaggtagtgaaaatagtaatcaataaatactgagggaactcagagaccggtgccagcgcgggtcctccgtatgctgagtgacggtcccttgggcccactgttccttctctatactttgtctctgtgtcttatttcttttctcagtctctcgtcccacctgacgagaaatacccacaggtgtggaggggctggacaccccttcgagccaggattatcagggcatttgggggtctgcaaaactaagccccaactcatcgatttcacaacttcatccagagccagcctgaacagtagttgcccatgatttctatgccttaatacgagaagagaacataggggctgggtgccaagtaggtagacagggagggcagggaactctaagacagagcttgaggggctcattcctcttgcaaaatgaaacaaaaaccacagcactgaatatgtaaatctcggtggctgaacccctcctaggatagtaagccctgacacaattgctgctatcttctctttctctcaaggaagtcaaaaaacacctgcagccttactgtccccttggaaacaagatgaacatctacattttctaaagtgggacaagaatctctgttcatatttatgtcccatgcatttgcacgtggccggacaaaggactttgcttctgccagcacatctgtcttcagatatgagaggaaacagacacaacctggaggcggcaaagaagcagctctttctcaagtgacctcctctatctccctacttcctggctaatggggcagccttgatccttgggaatccaggacagatatccactcgtgacaaactagctggaagaatgacaaccaatcaggttccaagcaccactggatgtgaaccacagaatttcctcctctccttgtggaatgtcagcttacgtctgacaaaaaatgtaaaactgagagagttacaatcttaaggaggagtcaagctaaagcagaaagaatcacctactctggactccagcatgactgctgagctcaaatatatatagagagagaaagaaccacaaacttgaagatggatatcagctacagactttcctgagtcaggtagggaaatggccatccctcaaaccttgcaaaaggcaaacttatgccattgtgtcctctgacatactgggtgatgtactgtatgttactgatgtgaggggaacttcctaaattggctagtaaattatgccaaataaaaagcaaaaatgatatttcttgaaatgttacatctgaggaacattgctaaaataatttatcagtagttttcaggatgatttatagatgtgcattgaagtgtgtacttgtgctctctctctcctctctctctctctttctctcctctctctcgctctttctctccttgcccccctccctccctgactttccttcctgtcccctccacagcagtttatattttttttctgataatctaactttgctgagggttcaatgtaaagcaccttcagtgatgagttagttggaatgttccccaagaaattctatttccagcactcttttacatgaaatccaagaagctctcagactatcttactgacaccttgcctttcctcaacagatcaatcttatcaatgtccatcacagatattttgtagaacggtggatcctggcagagtctcacagatgcttctgagacaacatttgctttcaaaaaatgaaccacacacatcctaaagatctcagccacttcccatgtttcattttgtgttacagcaaacatcacaacaatcattcctacagatcaccactgcatgtgatcaataaaatagtttttgcaacaatggtacttatgataatcatcttttattgtttacaaatactgctttacaatagttattcggttgcactgttcatattagatttccaattagctcacttaggaacataagtccctcgaacagctcagtcatctttttcattcctgtttctatcccctacatctctttcctttgcagacgactatctcctacactgaaacaggaaagcttttacctttttggcatgcttgatttaaagattatagaaaagtatttgacaaagaaaactcacacatgtgtgtacatatcttttaaaaagttatgtttatgcattgcacaggaatatcgagaatgctaataggcaatgtcagagtttactgtttttcaaaattagtacagttttattatttctaaaaactataaaatgaatatattcacatcaccatacagaagagtaggaggagatggcataaagtgtcattgttcctcctctgcaatcccaggagataactaccaagcacaatttatgtcttttaaaattcagcccgtatttatatacatatatattcaatgtagatgggatcatgatatctcaccacacatactcttcagtgacctgcattttcacaaacaccttccacgtaactatatagaagtctacgtcttccccttaatgtctgctttgtgctacattgtaaagctctagcacagtttaaccaaactcctattaatgaggattttagttatttttcactctttaaacaatatttccatgtgtagtcttatacatacgtctgtacacacttatcccagtctaaggagttccttttaccttcccccatcccagcattccctgtcacgcttgttgcttccgttgagtgactttactcctggagtataatctgcgtatagttcagttaaaaacatgggatctgagtttaggtcacagctctgccacttactgccataagccagttccttgacctctctgccctcaagtttttgcacctacaaagtaggggataatattagttcctagttcatagagtcttgggaataattaaatgtgatgatccatgtacaatgtctggcacttagtaagtgctcaataaatgtcaccctttatgattggtattgcgtgtatgtctgcagagaaaatcactttgtgtcccctttaaaaaaggactatgcccttggtcagctattttgcacattaaatttcacttgccaatattaactctccacctctaacttgatccctctccttcctcatcttctggtgagaccaaatgctaattctgctattcaaggcaactagcaaagctgccagtgacagaatcaaataaacctacccctaatctttagaattgtagttatgatttctgttgtaaaagttactgttgtggcagtcagtattagtctttggtctatgatagcatctctgatctattattgaytttcaattakgtatttttttttatttattctgaaaatgtttgttaagcatttgctaagtaaagatactggackgagcctcccaaatacagggcaaataaaacatcaaacagcttataatttagaagggtagaagagaatctgaaagcaggtaaaaataaacaggcactcggctgggcgcggtggctcacgcctgtaatcccagcactttgggaggccgaggtgggcggatcacgaggtcaggagatcgagaccatcctggctaacacggtgaaaccccgtctctactaaaaatacaaaaaattagcgaggcgtggtggcgggcgcctttagtcccagctagtcgggaggctgaggcaggagaatggtgtgaacccgggaggcggagcttgcagtgagccaagatcgcaccactgcactccagcctgggygacagagcgagactccgtctcaaaaaaaataaataaataaaataaaaaataattaggtactctaggcccagtgacctgtctctgtactctgtaaattcaggtcacctgctcagggctaatctgagagaaggtctctcttcagttgaattttgaaagacaattagcagttcacaagctaacccaggtggacaaagatgttcccaagcagagggagtgcttgtgaaagctggaggccatagaaaaactctaaggagtgtagggaggtgggagtaatgtatggaaggggtggagatggaaggttaagagagatacaaggctgcaaaaatggagctggactcaaaagaaaatactgaaaaggtcttcagtgttgttgatgagattactatggaaacactatggaacactgggactccatggcagctccaaagatggcatgcgcctggtccagctcagtaagagctgagctcttcctgtg

SEQ ID NO: 159 - DNA, 154 bp, Artificial Sequence
  synthetic
tctggcaacacggcctccctgaccgtctctgggctccaggctgaggatgaggctgattattactgcagctcatatgcaggcagcaacaatttaagtcttcggaactgggaccaaggtcaccgtcctaggtcagcccaagtccactcccactctc

SEQ ID NO: 160 - DNA, 156 bp, Artificial Sequence
  synthetic
tcagggacaatggccaccttgactatcagtggggcccaggtggaggatgaagctgactactactgttactcaacagacagcagtggtaatcattatgtcttcggaactgggaccaaggtcaccgtcctaggtcagcccaagtccactcccactctc

SEQ ID NO: 161 - DNA, 150 bp, Artificial Sequence
  synthetic
tctgggaacacagccactctgaccatcagcgggacccaggctatggatgaggctgactattactgtcaggcgtgggacagcagcactgccgtcttcggaactgggaccaaggtcaccgtcctaggtcagcccaagtccactcccactctc

SEQ ID NO: 162 - DNA, 21 bp, Artificial Sequence
  synthetic
aggtggaaacacggtgagagt

SEQ ID NO: 163 - DNA, 21 bp, Artificial Sequence
  synthetic
ccactcggggaaaagttggaa